European Patent Specification EP 3 749 372 B1, published April 16, 2025. Title: IL-12 antagonists with optimized linkers. Applicant: Philogen S.p.A. The sequence listing filed with the application follows.

SEQUENCE LISTING (36 sequences)

SEQ ID NO: 1 - protein, 306 aa, Homo sapiens
IWELKKDVYVVELDWYPDAPGEMVVLTCDTPEEDGITWTLDQSSEVLGSGKTLTIQVKEFGDAGQYTCHKGGEVLSHSLLLLHKKEDGIWSTDILKDQKEPKNKTFLRCEAKNYSGRFTCWWLTTISTDLTFSVKSSRGSSDPQGVTCGAATLSAERVRGDNKEYEYSVECQEDSACPAAEESLPIEVMVDAVHKLKYENYTSSFFIRDIIKPDPPKNLQLKPLKNSRQVEVSWEYPDTWSTPHSYFSLTFCVQVQGKSKREKKDRVFTDKTSATVICRKNASISVRAQDRYYSSSWSEWASVPCS

SEQ ID NO: 2 - protein, 15 aa, artificial sequence
  linker
GGGGSGGGGSGGGGS

SEQ ID NO: 3 - protein, 197 aa, Homo sapiens
RNLPVATPDPGMFPCLHHSQNLLRAVSNMLQKARQTLEFYPCTSEEIDHEDITKDKTSTVEACLPLELTKNESCLNSRETSFITNGSCLASRKTSFMMALCLSSIYEDLKMYQVEFKTMNAKLLMDPKRQIFLDQNMLAVIDELMQALNFNSETVPQKSSLEEPDFYKTKIKLCILLHAFRIRAVTIDRVMSYLNAS

SEQ ID NO: 4 - protein, 15 aa, artificial sequence
  linker
GSADGGSSAGGSDAG

SEQ ID NO: 5 - protein, 108 aa, artificial sequence [sequence omitted]

SEQ ID NO: 6 - protein, 5 aa, artificial sequence
  linker
GSSGG

SEQ ID NO: 7 - protein, 116 aa, artificial sequence [sequence omitted]

SEQ ID NO: 8 - protein, 15 aa, artificial sequence
  linker
SSSSGSSSSGSSSSG

SEQ ID NO: 9 - protein, 15 aa, artificial sequence
  linker
GGGAKGGGGKAGGGS

SEQ ID NO: 10 - protein, 15 aa, artificial sequence
  linker
GGGGDGGGGDGGGGS

SEQ ID NO: 11 - protein, 15 aa, artificial sequence
  linker
GGGGSGGGGSGGGGS

SEQ ID NO: 12 - protein, 15 aa, artificial sequence
  linker
GGGGSGGGGEGGGGS

SEQ ID NO: 13 - protein, 17 aa, artificial sequence
  linker
AEAAAKEAAAKEAAAKA

SEQ ID NO: 14 - protein, 12 aa, artificial sequence
  linker
APAPAPAPAPAP

SEQ ID NO: 15 - protein, 14 aa, artificial sequence
  linker
APAPAPAPAPAPAP

SEQ ID NO: 16 - protein, 1006 aa, artificial sequence
  Immunoconjugate sequence
IWELKKDVYVVELDWYPDAPGEMVVLTCDTPEEDGITWTLDQSSEVLGSGKTLTIQVKEFGDAGQYTCHKGGEVLSHSLLLLHKKEDGIWSTDILKDQKEPKNKTFLRCEAKNYSGRFTCWWLTTISTDLTFSVKSSRGSSDPQGVTCGAATLSAERVRGDNKEYEYSVECQEDSACPAAEESLPIEVMVDAVHKLKYENYTSSFFIRDIIKPDPPKNLQLKPLKNSRQVEVSWEYPDTWSTPHSYFSLTFCVQVQGKSKREKKDRVFTDKTSATVICRKNASISVRAQDRYYSSSWSEWASVPCSGGGGSGGGGSGGGGSRNLPVATPDPGMFPCLHHSQNLLRAVSNMLQKARQTLEFYPCTSEEIDHEDITKDKTSTVEACLPLELTKNESCLNSRETSFITNGSCLASRKTSFMMALCLSSIYEDLKMYQVEFKTMNAKLLMDPKRQIFLDQNMLAVIDELMQALNFNSETVPQKSSLEEPDFYKTKIKLCILLHAFRIRAVTIDRVMSYLNASGSADGGSSAGGSDAGEVQLLESGGGLVQPGGSLRLSCAASGFTFSSFSMSWVRQAPGKGLEWVSSISGSSGTTYYADSVKGRFTISRDNSKNTLYLQMNSLRAEDTAVYYCAKPFPYFDYWGQGTLVTVSSGSSGGEIVLTQSPGTLSLSPGERATLSCRASQSVSSSFLAWYQQKPGQAPRLLIYYASSRATGIPDRFSGSGSGTDFTLTISRLEPEDFAVYYCQQTGRIPPTFGQGTKVEIKSSSSGSSSSGSSSSGEVQLLESGGGLVQPGGSLRLSCAASGFTFSSFSMSWVRQAPGKGLEWVSSISGSSGTTYYADSVKGRFTISRDNSKNTLYLQMNSLRAEDTAVYYCAKPFPYFDYWGQGTLVTVSSGSSGGEIVLTQSPGTLSLSPGERATLSCRASQSVSSSFLAWYQQKPGQAPRLLIYYASSRATGIPDRFSGSGSGTDFTLTISRLEPEDFAVYYCQQTGRIPPTFGQGTKVEIK

SEQ ID NO: 17 - protein, 999 aa, artificial sequence
  Immunoconjugate sequence
MWELEKDVYVVEVDWTPDAPGETVNLTCDTPEEDDITWTSDQRHGVIGSGKTLTITVKEFLDAGQYTCHKGGETLSHSHLLLHKKENGIWSTEILKNFKNKTFLKCEAPNYSGRFTCSWLVQRNMDLKFNIKSSSSSPDSRAVTCGMASLSAEKVTLDQRDYEKYSVSCQEDVTCPTAEETLPIELALEARQQNKYENYSTSFFIRDIIKPDPPKNLQMRPLKNSQVEVSWEYPDSWSTPHSYFSLKFFVRIQRKKEKMKETEEGCNQKGAFLVERTSTEVQCKGGNVCVQAQDRYYNSSCSKWACVPCRVRSGGGGSGGGGSGGGGSRVIPVSGPARCLSQSRNLLKTTDDMVKTAREKLKHYSCTAEDIDHEDITRDQTSTLKTCLPLELHKNESCLATRETSSTTRGSCLPPQKTSLMMTLCLGSIYEDLKMYQTEFQAINAALQNHNHQQIILDKGMLVAIDELMQSLNHNGETLRQKPPVGEADPYRVKMKLCILLHAFSTRVVTINRVMGYLSSAGSADGEVQLLESGGGLVQPGGSLRLSCAASGFTFSSFSMSWVRQAPGKGLEWVSSISGSSGTTYYADSVKGRFTISRDNSKNTLYLQMNSLRAEDTAVYYCAKPFPYFDYWGQGTLVTVSSGSSGGEIVLTQSPGTLSLSPGERATLSCRASQSVSSSFLAWYQQKPGQAPRLLIYYASSRATGIPDRFSGSGSGTDFTLTISRLEPEDFAVYYCQQTGRIPPTFGQGTKVEIKSSSSGSSSSGSSSSGEVQLLESGGGLVQPGGSLRLSCAASGFTFSSFSMSWVRQAPGKGLEWVSSISGSSGTTYYADSVKGRFTISRDNSKNTLYLQMNSLRAEDTAVYYCAKPFPYFDYWGQGTLVTVSSGSSGGEIVLTQSPGTLSLSPGERATLSCRASQSVSSSFLAWYQQKPGQAPRLLIYYASSRATGIPDRFSGSGSGTDFTLTISRLEPEDFAVYYCQQTGRIPPTFGQGTKVEIK

SEQ ID NO: 18 - protein, 45 aa, artificial sequence
  linker
GGAGGGGGAGCTAAAGGTGGCGGTGGCAAGGCAGGGGGAGGGAGT

SEQ ID NO: 19 - DNA, 42 bp, artificial sequence
  linker
gcaccagcaccagcaccagcaccagcaccagcaccagcacca

SEQ ID NO: 20 - DNA, 45 bp, artificial sequence
  linker
ggaggtgggggtgatggtgggggaggtgacggcggaggtgggtct

SEQ ID NO: 21 - DNA, 36 bp, artificial sequence
  linker
gcaccagcaccagcaccagcaccagcaccagcacca

SEQ ID NO: 22 - DNA, 45 bp, artificial sequence
  linker
ggtggaggcgggtcaggcggagggggttctggcggtggcggatcg

SEQ ID NO: 23 - DNA, 45 bp, artificial sequence
  linker
ggtgggggtgggtccggaggcggaggcgaaggcggaggtgggtcg

SEQ ID NO: 24 - DNA, 51 bp, artificial sequence
  linker
gcagaagcagcagcaaaagaagcagcagcaaaagaagcagcagcaaaagca

SEQ ID NO: 25 - DNA, 45 bp, artificial sequence
  linker
gggtctgcagacggcggatcatcagctgggggaagtgacgcagga

SEQ ID NO: 26 - protein, 6 aa, artificial sequence
  linker
GSADGG

SEQ ID NO: 27 - protein, 997 aa, artificial sequence
  Immunoconjugate sequence
IWELKKDVYVVELDWYPDAPGEMVVLTCDTPEEDGITWTLDQSSEVLGSGKTLTIQVKEFGDAGQYTCHKGGEVLSHSLLLLHKKEDGIWSTDILKDQKEPKNKTFLRCEAKNYSGRFTCWWLTTISTDLTFSVKSSRGSSDPQGVTCGAATLSAERVRGDNKEYEYSVECQEDSACPAAEESLPIEVMVDAVHKLKYENYTSSFFIRDIIKPDPPKNLQLKPLKNSRQVEVSWEYPDTWSTPHSYFSLTFCVQVQGKSKREKKDRVFTDKTSATVICRKNASISVRAQDRYYSSSWSEWASVPCSGGGGSGGGGSGGGGSRNLPVATPDPGMFPCLHHSQNLLRAVSNMLQKARQTLEFYPCTSEEIDHEDITKDKTSTVEACLPLELTKNESCLNSRETSFITNGSCLASRKTSFMMALCLSSIYEDLKMYQVEFKTMNAKLLMDPKRQIFLDQNMLAVIDELMQALNFNSETVPQKSSLEEPDFYKTKIKLCILLHAFRIRAVTIDRVMSYLNASGSADGGEVQLLESGGGLVQPGGSLRLSCAASGFTFSSFSMSWVRQAPGKGLEWVSSISGSSGTTYYADSVKGRFTISRDNSKNTLYLQMNSLRAEDTAVYYCAKPFPYFDYWGQGTLVTVSSGSSGGEIVLTQSPGTLSLSPGERATLSCRASQSVSSSFLAWYQQKPGQAPRLLIYYASSRATGIPDRFSGSGSGTDFTLTISRLEPEDFAVYYCQQTGRIPPTFGQGTKVEIKSSSSGSSSSGSSSSGEVQLLESGGGLVQPGGSLRLSCAASGFTFSSFSMSWVRQAPGKGLEWVSSISGSSGTTYYADSVKGRFTISRDNSKNTLYLQMNSLRAEDTAVYYCAKPFPYFDYWGQGTLVTVSSGSSGGEIVLTQSPGTLSLSPGERATLSCRASQSVSSSFLAWYQQKPGQAPRLLIYYASSRATGIPDRFSGSGSGTDFTLTISRLEPEDFAVYYCQQTGRIPPTFGQGTKVEIK

SEQ ID NO: 28 - protein, 5 aa, artificial sequence
  antibody sequence (CDR)
SFSMS

SEQ ID NO: 29 - protein, 17 aa, artificial sequence
  antibody sequence (CDR)
SISGSSGTTYYADSVKG

SEQ ID NO: 30 - protein, 7 aa, artificial sequence
  antibody sequence (CDR)
PFPYFDY

SEQ ID NO: 31 - protein, 12 aa, artificial sequence
  antibody sequence (CDR)
RASQSVSSSFLA

SEQ ID NO: 32 - protein, 7 aa, artificial sequence
  antibody sequence (CDR)
YASSRAT

SEQ ID NO: 33 - protein, 9 aa, artificial sequence
  antibody sequence (CDR)
QQTGRIPPT

SEQ ID NO: 34 - protein, 5 aa, artificial sequence
  GGGGS linker
GGGGS

SEQ ID NO: 35 - protein, 5 aa, artificial sequence
  GGGGA linker
GGGGA

SEQ ID NO: 36 - protein, 229 aa, artificial sequence
  L19 Diabody
EVQLLESGGGLVQPGGSLRLSCAASGFTFSSFSMSWVRQAPGKGLEWVSSISGSSGTTYYADSVKGRFTISRDNSKNTLYLQMNSLRAEDTAVYYCAKPFPYFDYWGQGTLVTVSSGSSGGEIVLTQSPGTLSLSPGERATLSCRASQSVSSSFLAWYQQKPGQAPRLLIYYASSRATGIPDRFSGSGSGTDFTLTISRLEPEDFAVYYCQQTGRIPPTFGQGTKVEIK